European Patent Application EP 4 317 436 A1, published February 7, 2024. Title: A peptide from Norovirus, a polynucleotide, an antibody, a composition, and a method for identifying an epitope. Applicant: Denka Company Limited. The sequence listing filed with the application follows.

SEQUENCE LISTING (434 sequences)

SEQ ID NO: 1 - protein, 8 aa, Norovirus genogroup II
QVPDDHHQ

SEQ ID NO: 2 - protein, 8 aa, Norovirus genogroup II
RVPDDHHQ

SEQ ID NO: 3 - protein, 12 aa, Norovirus genogroup II
EVTAHLHDNEHL

SEQ ID NO: 4 - protein, 12 aa, Norovirus genogroup II
EVTAHLQDNDHL

SEQ ID NO: 5 - protein, 12 aa, Norovirus genogroup II
EVTAHLHDNDHL

SEQ ID NO: 6 - protein, 12 aa, Norovirus genogroup II
QVTAHLQDNEHL

SEQ ID NO: 7 - protein, 12 aa, Norovirus genogroup II
EVTAHLHDDDHL

SEQ ID NO: 8 - protein, 12 aa, Norovirus genogroup II
EVTAHLHDNGHL

SEQ ID NO: 9 - protein, 12 aa, Norovirus genogroup II
KVTAHLHDNDHL

SEQ ID NO: 10 - protein, 12 aa, Norovirus genogroup II
EVTTHLHDNDHL

SEQ ID NO: 11 - protein, 12 aa, Norovirus genogroup II
EVTAHLRDDEHL

SEQ ID NO: 12 - protein, 24 aa, Norovirus genogroup II
TLTRSTSRASDQADTATPRLFNYY

SEQ ID NO: 13 - protein, 24 aa, Norovirus genogroup II
TLTRSTSRAGDQADTATPRLFNYY

SEQ ID NO: 14 - protein, 24 aa, Norovirus genogroup II
TLTRSTSRTGDQADTASPRLFNYY

SEQ ID NO: 15 - protein, 24 aa, Norovirus genogroup II
TLTRSTNRVSDQADTATPRLFNYH

SEQ ID NO: 16 - protein, 24 aa, Norovirus genogroup II
TLTRSTNRASDQADTATPRLFNHH

SEQ ID NO: 17 - protein, 24 aa, Norovirus genogroup II
TLIRSTSRASDQADTSTPRLFNYY

SEQ ID NO: 18 - protein, 24 aa, Norovirus genogroup II
TLTRSTSRASDQADTPTPRLFNHR

SEQ ID NO: 19 - protein, 24 aa, Norovirus genogroup II
TLTRPTNRASDQADTATPRLFNHQ

SEQ ID NO: 20 - protein, 24 aa, Norovirus genogroup II
VLTRSTSRASDQADTATPRLFNYY

SEQ ID NO: 21 - protein, 24 aa, Norovirus genogroup II
VLTRSTSRTSDQADTATPRLFNYY

SEQ ID NO: 22 - protein, 24 aa, Norovirus genogroup II
VLTRSTSRASDQADTVTPRLFNYY

SEQ ID NO: 23 - protein, 24 aa, Norovirus genogroup II
VLTRSTSRASDQADAATPRLFNYY

SEQ ID NO: 24 - protein, 24 aa, Norovirus genogroup II
VLTRSTSRASDQADTATPRLFDYY

SEQ ID NO: 25 - protein, 24 aa, Norovirus genogroup II
VLTRSTSRASDHADTATPRLFNYY

SEQ ID NO: 26 - protein, 24 aa, Norovirus genogroup II
VLTRSTSRASDQADTAAPRLFNYY

SEQ ID NO: 27 - protein, 24 aa, Norovirus genogroup II
VMTRSTSRASDQADTAIPRLFNYY

SEQ ID NO: 28 - protein, 24 aa, Norovirus genogroup II
VLTRSTSRASDQADTATPRLFNYH

SEQ ID NO: 29 - protein, 24 aa, Norovirus genogroup II
MLTRSTSRASDQADTATPRLFNYY

SEQ ID NO: 30 - protein, 24 aa, Norovirus genogroup II
VLTRSTSRASDQADTAIPRLFNYY

SEQ ID NO: 31 - protein, 25 aa, Norovirus genogroup II
VLTQRTSRASDQADTAVTPRAFDHR

SEQ ID NO: 32 - protein, 24 aa, Norovirus genogroup II
VLTRSTSRASDQADAATPRLFNYH

SEQ ID NO: 33 - protein, 24 aa, Norovirus genogroup II
VLTRSTSRASDQSETTTPRLFNYY

SEQ ID NO: 34 - protein, 24 aa, Norovirus genogroup II
VLTRSTSRASDQADTTTPRLFNYY

SEQ ID NO: 35 - protein, 24 aa, Norovirus genogroup II
VLIRSTSRASDQADTATPRLFNYY

SEQ ID NO: 36 - protein, 24 aa, Norovirus genogroup II
VLTRSTSRASDQADAATPRLFNHY

SEQ ID NO: 37 - protein, 24 aa, Norovirus genogroup II
VLTRSTSRASDQADIATPRLFNYY

SEQ ID NO: 38 - protein, 24 aa, Norovirus genogroup II
VLTRSTSRASDQADTVTPRLFNHY

SEQ ID NO: 39 - protein, 24 aa, Norovirus genogroup II
VLTRSTSRANDQADTATPRFFDHS

SEQ ID NO: 40 - protein, 24 aa, Norovirus genogroup II
VLTRSTSRANDQADTATPRHFDLS

SEQ ID NO: 41 - protein, 24 aa, Norovirus genogroup II
VLIGSTSRASDQADTATPRSFNYY

SEQ ID NO: 42 - protein, 24 aa, Norovirus genogroup II
VLTRSTSRATDQADTATPRHFDHS

SEQ ID NO: 43 - protein, 24 aa, Norovirus genogroup II
VLTGSTSRASDQADTATPRLFNYY

SEQ ID NO: 44 - protein, 24 aa, Norovirus genogroup II
VLIGSTSRASDQADTATPRLFNYY

SEQ ID NO: 45 - protein, 24 aa, Norovirus genogroup II
VLTRSTSRANDQADTATPRHFGLS

SEQ ID NO: 46 - protein, 12 aa, Norovirus genogroup II
KVTGQVPNEQHM

SEQ ID NO: 47 - protein, 12 aa, Norovirus genogroup II
RITGQVPNEQHM

SEQ ID NO: 48 - protein, 22 aa, Norovirus genogroup II
IGQTSRSSDSTDSAPRRRDHPL

SEQ ID NO: 49 - protein, 22 aa, Norovirus genogroup II
ISQTARAADSTDSPQRARDHPL

SEQ ID NO: 50 - protein, 22 aa, Norovirus genogroup II
ISQTSRSAESTDSAPRVRNHPL

SEQ ID NO: 51 - protein, 22 aa, Norovirus genogroup II
ISQTARAADSTDSPQRARNHPL

SEQ ID NO: 52 - protein, 22 aa, Norovirus genogroup II
ISQTARATDSTDSPQRARDHPL

SEQ ID NO: 53 - protein, 22 aa, Norovirus genogroup II
ISQTARAADSVDSPQRARDHPL

SEQ ID NO: 54 - protein, 22 aa, Norovirus genogroup II
ISQTSRSADSTDSAPRVRNHPL

SEQ ID NO: 55 - protein, 22 aa, Norovirus genogroup II
VSQTSRSADSTDSAPRVRNHPL

SEQ ID NO: 56 - protein, 22 aa, Norovirus genogroup II
ISQAARAADSTDSPQRARDHPL

SEQ ID NO: 57 - protein, 22 aa, Norovirus genogroup II
ISQTARAVDSTDSPQRARDHPL

SEQ ID NO: 58 - protein, 22 aa, Norovirus genogroup II
IGQISRSSDSTDSAPRRRDHPL

SEQ ID NO: 59 - protein, 22 aa, Norovirus genogroup II
ISQTSRSADSTDSAPRVRNHPP

SEQ ID NO: 60 - protein, 22 aa, Norovirus genogroup II
ISQNARAADSPDSPQRARNHPL

SEQ ID NO: 61 - protein, 22 aa, Norovirus genogroup II
ISQNARAADLTDSPQRARNHPL

SEQ ID NO: 62 - protein, 22 aa, Norovirus genogroup II
ISQNARAADSTDSPQRARNHPL

SEQ ID NO: 63 - protein, 22 aa, Norovirus genogroup II
IGQTSRSPDSTDSAPRRRDHPL

SEQ ID NO: 64 - protein, 22 aa, Norovirus genogroup II
ISQTSRSADSIDSAPRVRNHPL

SEQ ID NO: 65 - protein, 22 aa, Norovirus genogroup II
ISQASRSADSTDSAPRVRNHPL

SEQ ID NO: 66 - protein, 22 aa, Norovirus genogroup II
ISQTSRSADSTDSAPRARNHPL

SEQ ID NO: 67 - protein, 22 aa, Norovirus genogroup II
ISQTSRSVDSTDSAPRARNHPL

SEQ ID NO: 68 - protein, 22 aa, Norovirus genogroup II
ISQTSRSADSTDSAQRVRNHPL

SEQ ID NO: 69 - protein, 22 aa, Norovirus genogroup II
ISQTSRSADSTDSAQRVRDHPL

SEQ ID NO: 70 - protein, 22 aa, Norovirus genogroup II
VSQTSRSADSTDSASRVRNHPL

SEQ ID NO: 71 - protein, 22 aa, Norovirus genogroup II
IGQTSRTSDSTDSAPRRRDHPL

SEQ ID NO: 72 - protein, 22 aa, Norovirus genogroup II
VSQTSRSADSTDSAPRVRSHPL

SEQ ID NO: 73 - protein, 22 aa, Norovirus genogroup II
ISQTSRSSDSTDSAPRRRDHPL

SEQ ID NO: 74 - protein, 7 aa, Norovirus genogroup II
GDVRSYR

SEQ ID NO: 75 - protein, 7 aa, Norovirus genogroup II
RDDRSYR

SEQ ID NO: 76 - protein, 11 aa, Norovirus genogroup II
INQKVSGENHV

SEQ ID NO: 77 - protein, 11 aa, Norovirus genogroup II
VNQKVSGENHV

SEQ ID NO: 78 - protein, 11 aa, Norovirus genogroup II
INQKVSGDNHV

SEQ ID NO: 79 - protein, 11 aa, Norovirus genogroup II
INQKVNGENHV

SEQ ID NO: 80 - protein, 12 aa, Norovirus genogroup II
VANNGDNWDQNL

SEQ ID NO: 81 - protein, 11 aa, Norovirus genogroup II
LANNDSWDQNL

SEQ ID NO: 82 - protein, 12 aa, Norovirus genogroup II
VANSGDNWDQNL

SEQ ID NO: 83 - protein, 12 aa, Norovirus genogroup II
VANSGDNWDQNV

SEQ ID NO: 84 - protein, 12 aa, Norovirus genogroup II
VANRGDNWDQNL

SEQ ID NO: 85 - protein, 12 aa, Norovirus genogroup II
VANHGDNWDQNL

SEQ ID NO: 86 - protein, 9 aa, Norovirus genogroup II
ELSDQPRYQ

SEQ ID NO: 87 - protein, 7 aa, Norovirus genogroup II
KLNEEPR

SEQ ID NO: 88 - protein, 7 aa, Norovirus genogroup II
KLSEEPR

SEQ ID NO: 89 - protein, 13 aa, Norovirus genogroup II
KLTADVHQSHDDR

SEQ ID NO: 90 - protein, 13 aa, Norovirus genogroup II
RLTADVDGSHDDR

SEQ ID NO: 91 - protein, 13 aa, Norovirus genogroup II
KISADVQNSHQDR

SEQ ID NO: 92 - protein, 11 aa, Norovirus genogroup II
RVTAQINQRDR

SEQ ID NO: 93 - protein, 11 aa, Norovirus genogroup II
RVTAETDHRDK

SEQ ID NO: 94 - protein, 11 aa, Norovirus genogroup II
RVTAKTDHRDK

SEQ ID NO: 95 - protein, 11 aa, Norovirus genogroup II
RVTTETDHRDK

SEQ ID NO: 96 - protein, 11 aa, Norovirus genogroup II
RVTAETDHHDK

SEQ ID NO: 97 - protein, 11 aa, Norovirus genogroup II
RVTAKTDHSDK

SEQ ID NO: 98 - protein, 11 aa, Norovirus genogroup II
RVTAETDNPDK

SEQ ID NO: 99 - protein, 13 aa, Norovirus genogroup II
KITADVRPSHDDR

SEQ ID NO: 100 - protein, 13 aa, Norovirus genogroup II
KITADVRPNHDDR

SEQ ID NO: 101 - protein, 11 aa, Norovirus genogroup II
RVTAETDHRDR

SEQ ID NO: 102 - protein, 11 aa, Norovirus genogroup II
RVTAQINQRDK

SEQ ID NO: 103 - protein, 11 aa, Norovirus genogroup II
RVTAQINQHDR

SEQ ID NO: 104 - protein, 11 aa, Norovirus genogroup II
RVTAQINQSDR

SEQ ID NO: 105 - protein, 11 aa, Norovirus genogroup II
RVTAEPSRSDR

SEQ ID NO: 106 - protein, 11 aa, Norovirus genogroup II
RVTAQINQCDR

SEQ ID NO: 107 - protein, 11 aa, Norovirus genogroup II
RVTAEVDQRDK

SEQ ID NO: 108 - protein, 12 aa, Norovirus genogroup II
ITSNPTSDYWDG

SEQ ID NO: 109 - protein, 12 aa, Norovirus genogroup II
TTSNDTSDYWDD

SEQ ID NO: 110 - protein, 12 aa, Norovirus genogroup II
MTSNPTSDYWDG

SEQ ID NO: 111 - protein, 12 aa, Norovirus genogroup II
MTSNPTSDYWDD

SEQ ID NO: 112 - protein, 12 aa, Norovirus genogroup II
TTSNPTSDYWDD

SEQ ID NO: 113 - protein, 12 aa, Norovirus genogroup II
STSNPTSDYWDD

SEQ ID NO: 114 - protein, 6 aa, Norovirus genogroup II
WSPKFT

SEQ ID NO: 115 - protein, 6 aa, Norovirus genogroup II
PTYTAQ

SEQ ID NO: 116 - protein, 6 aa, Norovirus genogroup II
PTYTPQ

SEQ ID NO: 117 - protein, 6 aa, Norovirus genogroup II
PTYTSQ

SEQ ID NO: 118 - protein, 6 aa, Norovirus genogroup II
PTYTAK

SEQ ID NO: 119 - protein, 6 aa, Norovirus genogroup II
PTYTTQ

SEQ ID NO: 120 - protein, 6 aa, Norovirus genogroup II
PTYAAQ

SEQ ID NO: 121 - protein, 6 aa, Norovirus genogroup II
PTHTAK

SEQ ID NO: 122 - protein, 8 aa, Norovirus genogroup II
DTTSGRFA

SEQ ID NO: 123 - protein, 8 aa, Norovirus genogroup II
DTTSGRFT

SEQ ID NO: 124 - protein, 8 aa, Norovirus genogroup II
DTTAGRFT

SEQ ID NO: 125 - protein, 8 aa, Norovirus genogroup II
DTASGRFT

SEQ ID NO: 126 - protein, 8 aa, Norovirus genogroup II
DTISGRFT

SEQ ID NO: 127 - protein, 8 aa, Norovirus genogroup II
DTTSSRFT

SEQ ID NO: 128 - protein, 8 aa, Norovirus genogroup II
DTSSPRFT

SEQ ID NO: 129 - protein, 8 aa, Norovirus genogroup II
DTTSPRFT

SEQ ID NO: 130 - protein, 8 aa, Norovirus genogroup II
DTKSGRFA

SEQ ID NO: 131 - protein, 8 aa, Norovirus genogroup II
NTTSGRFT

SEQ ID NO: 132 - protein, 8 aa, Norovirus genogroup II
DTTAGHFT

SEQ ID NO: 133 - protein, 6 aa, Norovirus genogroup II
YSDKYT

SEQ ID NO: 134 - protein, 6 aa, Norovirus genogroup II
TDPRYT

SEQ ID NO: 135 - protein, 6 aa, Norovirus genogroup II
TDPKYA

SEQ ID NO: 136 - protein, 6 aa, Norovirus genogroup II
TNPRYT

SEQ ID NO: 137 - protein, 6 aa, Norovirus genogroup II
TNPRYA

SEQ ID NO: 138 - protein, 6 aa, Norovirus genogroup II
KNPRYT

SEQ ID NO: 139 - protein, 6 aa, Norovirus genogroup II
TNSRYT

SEQ ID NO: 140 - protein, 6 aa, Norovirus genogroup II
TDPRYA

SEQ ID NO: 141 - protein, 6 aa, Norovirus genogroup II
GGDQYA

SEQ ID NO: 142 - protein, 6 aa, Norovirus genogroup II
GGNQYA

SEQ ID NO: 143 - protein, 6 aa, Norovirus genogroup II
NSAKFT

SEQ ID NO: 144 - protein, 6 aa, Norovirus genogroup II
NSTKFT

SEQ ID NO: 145 - protein, 6 aa, Norovirus genogroup II
DSAKFT

SEQ ID NO: 146 - protein, 6 aa, Norovirus genogroup II
DSTKFT

SEQ ID NO: 147 - protein, 6 aa, Norovirus genogroup II
HSTKFT

SEQ ID NO: 148 - protein, 6 aa, Norovirus genogroup II
TSGKFT

SEQ ID NO: 149 - protein, 6 aa, Norovirus genogroup II
TSGRFT

SEQ ID NO: 150 - protein, 6 aa, Norovirus genogroup II
AGDTFA

SEQ ID NO: 151 - protein, 9 aa, Norovirus genogroup II
STTSSQFVP

SEQ ID NO: 152 - protein, 9 aa, Norovirus genogroup II
ATTSTQFVP

SEQ ID NO: 153 - protein, 9 aa, Norovirus genogroup II
STYSPQFVP

SEQ ID NO: 154 - protein, 9 aa, Norovirus genogroup II
STHSPQFVP

SEQ ID NO: 155 - protein, 9 aa, Norovirus genogroup II
STYSPKFVP

SEQ ID NO: 156 - protein, 9 aa, Norovirus genogroup II
STYIPQFVP

SEQ ID NO: 157 - protein, 9 aa, Norovirus genogroup II
SPYSPQFVP

SEQ ID NO: 158 - protein, 9 aa, Norovirus genogroup II
STYSPQFVR

SEQ ID NO: 159 - protein, 6 aa, Norovirus genogroup II
TSEKFT

SEQ ID NO: 160 - protein, 6 aa, Norovirus genogroup II
TSDKFT

SEQ ID NO: 161 - protein, 8 aa, Norovirus genogroup II
GTWEESDL

SEQ ID NO: 162 - protein, 8 aa, Norovirus genogroup II
GTWEEHDL

SEQ ID NO: 163 - protein, 8 aa, Norovirus genogroup II
GAWEDRDF

SEQ ID NO: 164 - protein, 8 aa, Norovirus genogroup II
GTWEERDL

SEQ ID NO: 165 - protein, 8 aa, Norovirus genogroup II
GTWEDRDF

SEQ ID NO: 166 - protein, 8 aa, Norovirus genogroup II
GTWEEQDL

SEQ ID NO: 167 - protein, 14 aa, Norovirus genogroup II
IGTWQTDDLTVNQP

SEQ ID NO: 168 - protein, 14 aa, Norovirus genogroup II
IGTWQTDDLKVNQP

SEQ ID NO: 169 - protein, 14 aa, Norovirus genogroup II
IGTWQTDDITVDQP

SEQ ID NO: 170 - protein, 14 aa, Norovirus genogroup II
IGTWQTDDLQVNQP

SEQ ID NO: 171 - protein, 14 aa, Norovirus genogroup II
IGTWQTDDLTVSQP

SEQ ID NO: 172 - protein, 14 aa, Norovirus genogroup II
IGTWQTDDLTDNQP

SEQ ID NO: 173 - protein, 14 aa, Norovirus genogroup II
IGTWQTDDLTNNQP

SEQ ID NO: 174 - protein, 14 aa, Norovirus genogroup II
IGTWQTDDLAVNQP

SEQ ID NO: 175 - protein, 14 aa, Norovirus genogroup II
IGTWQTDDLTINQP

SEQ ID NO: 176 - protein, 14 aa, Norovirus genogroup II
IGTWQTNDLLDNQP

SEQ ID NO: 177 - protein, 14 aa, Norovirus genogroup II
IGTWQTDDLTVNQS

SEQ ID NO: 178 - protein, 14 aa, Norovirus genogroup II
IGTWQIDDLTVNQP

SEQ ID NO: 179 - protein, 14 aa, Norovirus genogroup II
IGTWQTDDLIVNQP

SEQ ID NO: 180 - protein, 14 aa, Norovirus genogroup II
IGTWQTDDITVNQP

SEQ ID NO: 181 - protein, 14 aa, Norovirus genogroup II
IGTWQTDDLNVNQP

SEQ ID NO: 182 - protein, 14 aa, Norovirus genogroup II
VGTWQTDDLTVNQP

SEQ ID NO: 183 - protein, 13 aa, Norovirus genogroup II
ISTESSDFDSNQP

SEQ ID NO: 184 - protein, 13 aa, Norovirus genogroup II
ISTESGDFDPNQP

SEQ ID NO: 185 - protein, 13 aa, Norovirus genogroup II
ISTESDDFDPNQP

SEQ ID NO: 186 - protein, 13 aa, Norovirus genogroup II
ISTESDDFDSNQP

SEQ ID NO: 187 - protein, 13 aa, Norovirus genogroup II
ITTESNDFDSNQP

SEQ ID NO: 188 - protein, 13 aa, Norovirus genogroup II
ITTESDDFDPNQS

SEQ ID NO: 189 - protein, 13 aa, Norovirus genogroup II
IITESDDFDLNQS

SEQ ID NO: 190 - protein, 13 aa, Norovirus genogroup II
ISTETDDFNQNQP

SEQ ID NO: 191 - protein, 13 aa, Norovirus genogroup II
ITTESDDFDTNQS

SEQ ID NO: 192 - protein, 13 aa, Norovirus genogroup II
ITTESDDFNQNKP

SEQ ID NO: 193 - protein, 13 aa, Norovirus genogroup II
ISTESDDFDQNQP

SEQ ID NO: 194 - protein, 13 aa, Norovirus genogroup II
ISTESGDFDQNQP

SEQ ID NO: 195 - protein, 13 aa, Norovirus genogroup II
ISTESDDFHQNQP

SEQ ID NO: 196 - protein, 13 aa, Norovirus genogroup II
ISTESDDFDQNKP

SEQ ID NO: 197 - protein, 13 aa, Norovirus genogroup II
ISTESDDFDQNQS

SEQ ID NO: 198 - protein, 13 aa, Norovirus genogroup II
ISTESDDFDENKP

SEQ ID NO: 199 - protein, 13 aa, Norovirus genogroup II
MSTESDDFDQNQP

SEQ ID NO: 200 - protein, 13 aa, Norovirus genogroup II
ISTESSDFDQNQP

SEQ ID NO: 201 - protein, 13 aa, Norovirus genogroup II
ISTESGDFEQNQP

SEQ ID NO: 202 - protein, 13 aa, Norovirus genogroup II
ISTESDDFDENQP

SEQ ID NO: 203 - protein, 13 aa, Norovirus genogroup II
MSTESSDFDQNQP

SEQ ID NO: 204 - protein, 13 aa, Norovirus genogroup II
ISTESDDFAQNQP

SEQ ID NO: 205 - protein, 13 aa, Norovirus genogroup II
ISTESDDFEHNQP

SEQ ID NO: 206 - protein, 13 aa, Norovirus genogroup II
ISTESDDFEQNQP

SEQ ID NO: 207 - protein, 13 aa, Norovirus genogroup II
ISTESGDFDQNKP

SEQ ID NO: 208 - protein, 13 aa, Norovirus genogroup II
ISTESHDFDENEP

SEQ ID NO: 209 - protein, 13 aa, Norovirus genogroup II
ISTESSDFDQSQP

SEQ ID NO: 210 - protein, 13 aa, Norovirus genogroup II
ISTESHDFDQNEP

SEQ ID NO: 211 - protein, 13 aa, Norovirus genogroup II
ISTESGDFDQNEP

SEQ ID NO: 212 - protein, 13 aa, Norovirus genogroup II
ISTESDDFNQNQP

SEQ ID NO: 213 - protein, 13 aa, Norovirus genogroup II
ISTESDDFELNQP

SEQ ID NO: 214 - protein, 6 aa, Norovirus genogroup II
GTWNTN

SEQ ID NO: 215 - protein, 11 aa, Norovirus genogroup II
MHSESDDFVTG

SEQ ID NO: 216 - protein, 11 aa, Norovirus genogroup II
IKSESNDFTTN

SEQ ID NO: 217 - protein, 11 aa, Norovirus genogroup II
MYSESTDFDDG

SEQ ID NO: 218 - protein, 11 aa, Norovirus genogroup II
IKSGSDDFNTN

SEQ ID NO: 219 - protein, 11 aa, Norovirus genogroup II
IKSESNDFITN

SEQ ID NO: 220 - protein, 11 aa, Norovirus genogroup II
IKSDSNDFNTN

SEQ ID NO: 221 - protein, 11 aa, Norovirus genogroup II
MHSESSDFDDG

SEQ ID NO: 222 - protein, 11 aa, Norovirus genogroup II
MNSESSDFDDG

SEQ ID NO: 223 - protein, 11 aa, Norovirus genogroup II
MYSESSDFDDG

SEQ ID NO: 224 - protein, 11 aa, Norovirus genogroup II
IKSESTDFTTN

SEQ ID NO: 225 - protein, 11 aa, Norovirus genogroup II
IKSESPDFNTN

SEQ ID NO: 226 - protein, 11 aa, Norovirus genogroup II
MRSESDDFVTG

SEQ ID NO: 227 - protein, 11 aa, Norovirus genogroup II
MHSESGDFVTG

SEQ ID NO: 228 - protein, 11 aa, Norovirus genogroup II
IHSESDDFVTG

SEQ ID NO: 229 - protein, 11 aa, Norovirus genogroup II
MYSESDDFDDG

SEQ ID NO: 230 - protein, 11 aa, Norovirus genogroup II
IKSESTDFTTS

SEQ ID NO: 231 - protein, 11 aa, Norovirus genogroup II
MYSESDDFVTG

SEQ ID NO: 232 - protein, 11 aa, Norovirus genogroup II
MHSESTDFDDG

SEQ ID NO: 233 - protein, 11 aa, Norovirus genogroup II
MYSESNDFDDG

SEQ ID NO: 234 - protein, 11 aa, Norovirus genogroup II
MYSESDDFDNG

SEQ ID NO: 235 - protein, 11 aa, Norovirus genogroup II
MYSESGDFDDG

SEQ ID NO: 236 - protein, 11 aa, Norovirus genogroup II
MYSESPDFDDG

SEQ ID NO: 237 - protein, 11 aa, Norovirus genogroup II
MYSESEDFVTG

SEQ ID NO: 238 - protein, 11 aa, Norovirus genogroup II
IKSESPDFTTN

SEQ ID NO: 239 - protein, 9 aa, Norovirus genogroup II
FSESQDFEV

SEQ ID NO: 240 - protein, 9 aa, Norovirus genogroup II
FSESDDFDE

SEQ ID NO: 241 - protein, 6 aa, Norovirus genogroup II
GTWEED

SEQ ID NO: 242 - protein, 6 aa, Norovirus genogroup II
GTWEQD

SEQ ID NO: 243 - protein, 6 aa, Norovirus genogroup II
GTWEEN

SEQ ID NO: 244 - protein, 9 aa, Norovirus genogroup II
HSITEHVHP

SEQ ID NO: 245 - protein, 9 aa, Norovirus genogroup II
HSITGDVHH

SEQ ID NO: 246 - protein, 9 aa, Norovirus genogroup II
HSITENVHP

SEQ ID NO: 247 - protein, 9 aa, Norovirus genogroup II
HSITEDVRP

SEQ ID NO: 248 - protein, 6 aa, Norovirus genogroup II
KSSSND

SEQ ID NO: 249 - protein, 6 aa, Norovirus genogroup II
KSSSSD

SEQ ID NO: 250 - protein, 13 aa, Norovirus genogroup II
FGSTSDDFQLQQP

SEQ ID NO: 251 - protein, 13 aa, Norovirus genogroup II
FGSTSTDFQLQQP

SEQ ID NO: 252 - protein, 13 aa, Norovirus genogroup II
FGSESEDFQVGPP

SEQ ID NO: 253 - protein, 13 aa, Norovirus genogroup II
LRISDNDDFQFQP

SEQ ID NO: 254 - protein, 12 aa, Norovirus genogroup II
FRSNDNDFQLQP

SEQ ID NO: 255 - protein, 12 aa, Norovirus genogroup II
FRSNDDDFQLQP

SEQ ID NO: 256 - protein, 13 aa, Norovirus genogroup II
FGSTSEDFIVGQP

SEQ ID NO: 257 - protein, 13 aa, Norovirus genogroup II
LRISDNDDFQFHP

SEQ ID NO: 258 - protein, 12 aa, Norovirus genogroup II
FRSNDDDFQWQP

SEQ ID NO: 259 - protein, 13 aa, Norovirus genogroup II
LRISNNDDFQFQP

SEQ ID NO: 260 - protein, 12 aa, Norovirus genogroup II
FGSNDNDFQLQP

SEQ ID NO: 261 - protein, 13 aa, Norovirus genogroup II
FRISDNDDFQFQP

SEQ ID NO: 262 - protein, 13 aa, Norovirus genogroup II
LRISDNDDFQLQP

SEQ ID NO: 263 - protein, 13 aa, Norovirus genogroup II
FKISSDDDFQLQP

SEQ ID NO: 264 - protein, 13 aa, Norovirus genogroup II
LRISDNNDFQFQP

SEQ ID NO: 265 - protein, 13 aa, Norovirus genogroup II
FRISNNDDFQFQP

SEQ ID NO: 266 - protein, 7 aa, Norovirus genogroup II
HQVQGDI

SEQ ID NO: 267 - protein, 7 aa, Norovirus genogroup II
HQVQGDT

SEQ ID NO: 268 - protein, 5 aa, Norovirus genogroup II
FNTDH

SEQ ID NO: 269 - protein, 5 aa, Norovirus genogroup II
YDTGH

SEQ ID NO: 270 - protein, 5 aa, Norovirus genogroup II
YDTNH

SEQ ID NO: 271 - protein, 5 aa, Norovirus genogroup II
YDTEH

SEQ ID NO: 272 - protein, 8 aa, Norovirus genogroup II
LNDVEHFN

SEQ ID NO: 273 - protein, 8 aa, Norovirus genogroup II
LNDTEHFN

SEQ ID NO: 274 - protein, 8 aa, Norovirus genogroup II
LNDTDHFN

SEQ ID NO: 275 - protein, 8 aa, Norovirus genogroup II
LSDTDHSN

SEQ ID NO: 276 - protein, 8 aa, Norovirus genogroup II
LSDTDHFN

SEQ ID NO: 277 - protein, 8 aa, Norovirus genogroup II
LNDIEHFN

SEQ ID NO: 278 - protein, 8 aa, Norovirus genogroup II
LNDTEHFD

SEQ ID NO: 279 - protein, 8 aa, Norovirus genogroup II
LNDTDHFD

SEQ ID NO: 280 - protein, 8 aa, Norovirus genogroup II
LNDTGHFN

SEQ ID NO: 281 - protein, 8 aa, Norovirus genogroup II
LNDTEYFN

SEQ ID NO: 282 - protein, 8 aa, Norovirus genogroup II
LNDTEHLN

SEQ ID NO: 283 - protein, 8 aa, Norovirus genogroup II
LNDNEHFN

SEQ ID NO: 284 - protein, 8 aa, Norovirus genogroup II
FNDTEHFN

SEQ ID NO: 285 - protein, 8 aa, Norovirus genogroup II
LNDAEHFN

SEQ ID NO: 286 - protein, 7 aa, Norovirus genogroup II
DNEADFQ

SEQ ID NO: 287 - protein, 7 aa, Norovirus genogroup II
DRETDFQ

SEQ ID NO: 288 - protein, 7 aa, Norovirus genogroup II
DNEVDFQ

SEQ ID NO: 289 - protein, 7 aa, Norovirus genogroup II
DNEAEFQ

SEQ ID NO: 290 - protein, 7 aa, Norovirus genogroup II
DREADFQ

SEQ ID NO: 291 - protein, 7 aa, Norovirus genogroup II
DHEADFQ

SEQ ID NO: 292 - protein, 7 aa, Norovirus genogroup II
DHEEDFQ

SEQ ID NO: 293 - protein, 7 aa, Norovirus genogroup II
DREVDFQ

SEQ ID NO: 294 - protein, 7 aa, Norovirus genogroup II
DHEVDFQ

SEQ ID NO: 295 - protein, 7 aa, Norovirus genogroup II
DQEADFQ

SEQ ID NO: 296 - protein, 7 aa, Norovirus genogroup II
DHETDFQ

SEQ ID NO: 297 - protein, 7 aa, Norovirus genogroup II
DHESDFQ

SEQ ID NO: 298 - protein, 7 aa, Norovirus genogroup II
DNEREFQ

SEQ ID NO: 299 - protein, 7 aa, Norovirus genogroup II
DHEPDFQ

SEQ ID NO: 300 - protein, 7 aa, Norovirus genogroup II
DHEEHFQ

SEQ ID NO: 301 - protein, 7 aa, Norovirus genogroup II
DHEEDFK

SEQ ID NO: 302 - protein, 7 aa, Norovirus genogroup II
DREADFE

SEQ ID NO: 303 - protein, 7 aa, Norovirus genogroup II
DHEEDFR

SEQ ID NO: 304 - protein, 7 aa, Norovirus genogroup II
DNEAHFK

SEQ ID NO: 305 - protein, 7 aa, Norovirus genogroup II
DSEADFQ

SEQ ID NO: 306 - protein, 7 aa, Norovirus genogroup II
DQESDFQ

SEQ ID NO: 307 - protein, 6 aa, Norovirus genogroup II
VANGHR

SEQ ID NO: 308 - protein, 6 aa, Norovirus genogroup II
VSDGHR

SEQ ID NO: 309 - protein, 5 aa, Norovirus genogroup II
DNDWH

SEQ ID NO: 310 - protein, 5 aa, Norovirus genogroup II
DNNWR

SEQ ID NO: 311 - protein, 5 aa, Norovirus genogroup II
ADDWR

SEQ ID NO: 312 - protein, 5 aa, Norovirus genogroup II
ADDWH

SEQ ID NO: 313 - protein, 5 aa, Norovirus genogroup II
DDDWH

SEQ ID NO: 314 - protein, 5 aa, Norovirus genogroup II
DDDWR

SEQ ID NO: 315 - protein, 5 aa, Norovirus genogroup II
DTSHP

SEQ ID NO: 316 - protein, 5 aa, Norovirus genogroup II
DDSHP

SEQ ID NO: 317 - protein, 5 aa, Norovirus genogroup II
DASHP

SEQ ID NO: 318 - protein, 5 aa, Norovirus genogroup II
DPSHP

SEQ ID NO: 319 - protein, 5 aa, Norovirus genogroup II
DNSHP

SEQ ID NO: 320 - protein, 6 aa, Norovirus genogroup II
EHEDFS

SEQ ID NO: 321 - protein, 6 aa, Norovirus genogroup II
ENEGFN

SEQ ID NO: 322 - protein, 6 aa, Norovirus genogroup II
DTDDFN

SEQ ID NO: 323 - protein, 6 aa, Norovirus genogroup II
EDEGFN

SEQ ID NO: 324 - protein, 6 aa, Norovirus genogroup II
ESEGFN

SEQ ID NO: 325 - protein, 6 aa, Norovirus genogroup II
EREGFN

SEQ ID NO: 326 - protein, 8 aa, Norovirus genogroup II
VNENTPFQ

SEQ ID NO: 327 - protein, 8 aa, Norovirus genogroup II
VNENTPFK

SEQ ID NO: 328 - protein, 8 aa, Norovirus genogroup II
QNENTPFQ

SEQ ID NO: 329 - protein, 7 aa, Norovirus genogroup II
DDQHPFR

SEQ ID NO: 330 - protein, 7 aa, Norovirus genogroup II
DDQHPFK

SEQ ID NO: 331 - protein, 11 aa, Norovirus genogroup II
GIKVESGHDFD

SEQ ID NO: 332 - protein, 11 aa, Norovirus genogroup II
GIKIESGHEFD

SEQ ID NO: 333 - protein, 11 aa, Norovirus genogroup II
GIKIETGHSFR

SEQ ID NO: 334 - protein, 12 aa, Norovirus genogroup II
GVNDDDDGHPFR

SEQ ID NO: 335 - protein, 11 aa, Norovirus genogroup II
GINDDGDHPFR

SEQ ID NO: 336 - protein, 11 aa, Norovirus genogroup II
GINDDDDHPFR

SEQ ID NO: 337 - protein, 12 aa, Norovirus genogroup II
GVNDDDDGHTFR

SEQ ID NO: 338 - protein, 11 aa, Norovirus genogroup II
CINDDDDHPFR

SEQ ID NO: 339 - protein, 11 aa, Norovirus genogroup II
GINDDGNHPFR

SEQ ID NO: 340 - protein, 11 aa, Norovirus genogroup II
GIKIEDGHAFD

SEQ ID NO: 341 - protein, 12 aa, Norovirus genogroup II
GVNDDNDGPPFR

SEQ ID NO: 342 - protein, 12 aa, Norovirus genogroup II
GVNDDDDGHSFR

SEQ ID NO: 343 - protein, 12 aa, Norovirus genogroup II
GVNDDDDGNPFR

SEQ ID NO: 344 - protein, 12 aa, Norovirus genogroup II
GVNDDDGGHPFR

SEQ ID NO: 345 - protein, 11 aa, Norovirus genogroup II
GVNDDDGHPFR

SEQ ID NO: 346 - protein, 12 aa, Norovirus genogroup II
AINEEDDDHPFR

SEQ ID NO: 347 - protein, 12 aa, Norovirus genogroup II
SVNDDDDGHPFR

SEQ ID NO: 348 - protein, 12 aa, Norovirus genogroup II
GVNDDDDDHPFR

SEQ ID NO: 349 - protein, 13 aa, Norovirus genogroup II
GVNDDDDGGRPFR

SEQ ID NO: 350 - protein, 7 aa, Norovirus genogroup II
NGNTPFR

SEQ ID NO: 351 - protein, 7 aa, Norovirus genogroup II
NQNTPFK

SEQ ID NO: 352 - protein, 7 aa, Norovirus genogroup II
SYSGRLT

SEQ ID NO: 353 - protein, 7 aa, Norovirus genogroup II
NYSGRLT

SEQ ID NO: 354 - protein, 7 aa, Norovirus genogroup II
RYAGALN

SEQ ID NO: 355 - protein, 7 aa, Norovirus genogroup II
KYAGALN

SEQ ID NO: 356 - protein, 7 aa, Norovirus genogroup II
RFAGALN

SEQ ID NO: 357 - protein, 7 aa, Norovirus genogroup II
GYAGALN

SEQ ID NO: 358 - protein, 7 aa, Norovirus genogroup II
DYSGQFT

SEQ ID NO: 359 - protein, 7 aa, Norovirus genogroup II
EYSGQFT

SEQ ID NO: 360 - protein, 7 aa, Norovirus genogroup II
DYSGQLT

SEQ ID NO: 361 - protein, 7 aa, Norovirus genogroup II
NYSGQFT

SEQ ID NO: 362 - protein, 7 aa, Norovirus genogroup II
DYAGQFT

SEQ ID NO: 363 - protein, 7 aa, Norovirus genogroup II
NYAGQFT

SEQ ID NO: 364 - protein, 7 aa, Norovirus genogroup II
DYAGQLT

SEQ ID NO: 365 - protein, 7 aa, Norovirus genogroup II
DYAGQIT

SEQ ID NO: 366 - protein, 7 aa, Norovirus genogroup II
NYAGQLT

SEQ ID NO: 367 - protein, 7 aa, Norovirus genogroup II
NYAGQIS

SEQ ID NO: 368 - protein, 7 aa, Norovirus genogroup II
NYAGQIT

SEQ ID NO: 369 - protein, 7 aa, Norovirus genogroup II
RYSGALT

SEQ ID NO: 370 - protein, 7 aa, Norovirus genogroup II
DYSGHLT

SEQ ID NO: 371 - protein, 7 aa, Norovirus genogroup II
DYSGRLT

SEQ ID NO: 372 - protein, 7 aa, Norovirus genogroup II
EYSGHLT

SEQ ID NO: 373 - protein, 7 aa, Norovirus genogroup II
DYSGSLT

SEQ ID NO: 374 - protein, 7 aa, Norovirus genogroup II
DYPGHLT

SEQ ID NO: 375 - protein, 7 aa, Norovirus genogroup II
RYGGHLT

SEQ ID NO: 376 - protein, 7 aa, Norovirus genogroup II
NYSGALT

SEQ ID NO: 377 - protein, 7 aa, Norovirus genogroup II
HYAGSLA

SEQ ID NO: 378 - protein, 7 aa, Norovirus genogroup II
HYSGSLA

SEQ ID NO: 379 - protein, 7 aa, Norovirus genogroup II
HYAGALA

SEQ ID NO: 380 - protein, 7 aa, Norovirus genogroup II
HYARALA

SEQ ID NO: 381 - protein, 7 aa, Norovirus genogroup II
NYGGHLA

SEQ ID NO: 382 - protein, 8 aa, Norovirus genogroup II
RYSGHLTL

SEQ ID NO: 383 - protein, 8 aa, Norovirus genogroup II
NYSGALTL

SEQ ID NO: 384 - protein, 8 aa, Norovirus genogroup II
NYSGELTL

SEQ ID NO: 385 - protein, 8 aa, Norovirus genogroup II
DYSGLLTL

SEQ ID NO: 386 - protein, 8 aa, Norovirus genogroup II
DYSGPLTL

SEQ ID NO: 387 - protein, 8 aa, Norovirus genogroup II
DYSGVLTL

SEQ ID NO: 388 - protein, 8 aa, Norovirus genogroup II
NYSGELTS

SEQ ID NO: 389 - protein, 8 aa, Norovirus genogroup II
NYSGEFTL

SEQ ID NO: 390 - protein, 8 aa, Norovirus genogroup II
SYSGELTL

SEQ ID NO: 391 - protein, 6 aa, Norovirus genogroup II
DFLANI

SEQ ID NO: 392 - protein, 6 aa, Norovirus genogroup II
DFQGRV

SEQ ID NO: 393 - protein, 6 aa, Norovirus genogroup II
DFEGRV

SEQ ID NO: 394 - protein, 6 aa, Norovirus genogroup II
DFQGKV

SEQ ID NO: 395 - protein, 6 aa, Norovirus genogroup II
DFQGRI

SEQ ID NO: 396 - protein, 6 aa, Norovirus genogroup II
DFQERV

SEQ ID NO: 397 - protein, 6 aa, Norovirus genogroup II
DFRGKV

SEQ ID NO: 398 - protein, 6 aa, Norovirus genogroup II
DFRGKI

SEQ ID NO: 399 - protein, 6 aa, Norovirus genogroup II
DFRGRV

SEQ ID NO: 400 - protein, 6 aa, Norovirus genogroup II
DFHGKV

SEQ ID NO: 401 - protein, 6 aa, Norovirus genogroup II
DFAGEV

SEQ ID NO: 402 - protein, 6 aa, Norovirus genogroup II
DFKGAV

SEQ ID NO: 403 - protein, 6 aa, Norovirus genogroup II
DFKGTV

SEQ ID NO: 404 - protein, 6 aa, Norovirus genogroup II
DFRGIL

SEQ ID NO: 405 - protein, 6 aa, Norovirus genogroup II
DFQGIL

SEQ ID NO: 406 - protein, 6 aa, Norovirus genogroup II
DFSGKL

SEQ ID NO: 407 - protein, 6 aa, Norovirus genogroup II
DFSGRL

SEQ ID NO: 408 - protein, 6 aa, Norovirus genogroup II
DFSGML

SEQ ID NO: 409 - protein, 6 aa, Norovirus genogroup II
DFSGIL

SEQ ID NO: 410 - protein, 6 aa, Norovirus genogroup II
DFSGLL

SEQ ID NO: 411 - protein, 6 aa, Norovirus genogroup II
DFQAML

SEQ ID NO: 412 - protein, 6 aa, Norovirus genogroup II
DFQAVL

SEQ ID NO: 413 - protein, 6 aa, Norovirus genogroup II
DFTGLL

SEQ ID NO: 414 - protein, 6 aa, Norovirus genogroup II
DFKGVV

SEQ ID NO: 415 - protein, 6 aa, Norovirus genogroup II
DFKGFV

SEQ ID NO: 416 - protein, 4 aa, Norovirus genogroup II
QWAL

SEQ ID NO: 417 - protein, 4 aa, Norovirus genogroup II
QWVL

SEQ ID NO: 418 - protein, 4 aa, Norovirus genogroup II
QWIL

SEQ ID NO: 419 - protein, 4 aa, Norovirus genogroup II
QWVV

SEQ ID NO: 420 - protein, 4 aa, Norovirus genogroup II
QWMV

SEQ ID NO: 421 - protein, 4 aa, Norovirus genogroup II
QWAV

SEQ ID NO: 422 - protein, 4 aa, Norovirus genogroup II
QWTL

SEQ ID NO: 423 - protein, 4 aa, Norovirus genogroup II
QWSL

SEQ ID NO: 424 - protein, 4 aa, Norovirus genogroup II
QWEL

SEQ ID NO: 425 - protein, 4 aa, Norovirus genogroup II
QWDP

SEQ ID NO: 426 - protein, 10 aa, Norovirus genogroup II
GMGADDWHQW

SEQ ID NO: 427 - protein, 11 aa, Norovirus genogroup II
PEYSGHLTLNM

SEQ ID NO: 428 - protein, 15 aa, Norovirus genogroup II
NLRISDNDDFQFQPT

SEQ ID NO: 429 - protein, 16 aa, Norovirus genogroup II
PVGVNDDDDGHPFRQW

SEQ ID NO: 430 - protein, 10 aa, Norovirus genogroup II
PNYSGELTLN

SEQ ID NO: 431 - protein, 11 aa, Norovirus genogroup II
GLNDTEHFNQW

SEQ ID NO: 432 - DNA, 1629 bp, Norovirus GII.2
atgaagatggcgtcgaatgacgccgctccatctactgatggtgcagccggcctcgtgccagaaagtaataatgaggtcatggctcttgaacccgtggctggcgccgccttggcagccccggtcaccggtcaaacaaatattatagacccttggattagagcaaattttgtccaggcccctaatggtgaatttacagtctctccccgtaatgcccctggtgaagtgctattgaatctagagttgggtccagaattaaatccttatctggcacatttagcaagaatgtacaacgggtatgccggtgggatggaggtgcaggtcatgttggctgggaacgcgttcacagccggcaagttggtcttcgccgctgtgccacctcacttcccggttgaaaaccttagtccacagcaaattaccatgttccctcatgtgattatagatgtaaggactttggaacctgttttattaccactccctgatgttagaaataatttcttccattataatcagaaagatgatcccaagatgagaattgtggctatgctttataccccccttaggtctaatggttcaggtgatgatgtgtttacagtctcctgcagggtgttgactagaccctcccctgattttgatttcacatatctggtgccaccaacagtggagtctaaaacaaaaccatttaccctcccaatcctcacacttggggaactttccaattctagattcccagtgtccatagaccagatgtacaccagccccaatgaagttatatcagtgcagtgtcaaaatggtaggtgcacactggatggggagctccaaggaacaacacaactccaagtcagtggtatttgtgctttcaagggagaagtgaccgcccatttgcatgacaatgatcatctatataatgtcaccatcacaaacttgaatgggtccccctttgacccctccgaggacatccctgcccctctgggcgtacctgactttcagggaagggtctttggtgtcatctcccaaagagacaaacacaattcccctggacataatgaaccagcaaatagggggcacgacgctgtggtccctacttacacatcacagtacactccaaaattgggtcagattcaaattggcacatggcaaaccgatgatcttacagtcaaccaaccagtcaaattcaccccagttggactcaatgacactgaacattttaaccaatgggtggtccccagatatgctggtgctctaaaccttaacacaaaccttgccccttctgttgctccagtatttccaggggagcgcctgctctttttcagatcatacatccccctcaagggtggttatggaaatccagccattgattgcctactaccacaagagtgggtgcagcatttctatcaggaagcagccccttcaatgagtgaggtggcccttgtcagatacatcaacccggatactggtcgggcactgtttgaggccaagctccacagagctggtttcatgacagtctcaagcaacaccagtgccccggtggttgtgcctgccaacggatacttcagatttgattcttgggtgaaccaattctattctctcgcccccatgggaactggaaatgggcgtagaagggttcaataa

SEQ ID NO: 433 - DNA, 2476 bp, Norovirus GII.6
gtgaatgaagatggcgtcgaatgacgctgctccatcgaatgatggtgctgccaacctcgtaccagaggccaacaatgaggttatggcacttgaaccggtggtgggagcctcaattgcagctcctgtcgtcggtcaacagaatataattgacccctggattagagaaaattttgttcaggcaccacagggtgagtttactgtttcaccaagaaactcgcctggtgagatgcttttaaatcttgaattaggcccagagctcaatccttacttgagtcatttgtcccgcatgtacaatggttatgctggtggcatgcaggttcaggtggtcctagctgggaatgcgttcacagctggtaaaatcatctttgccgccgttccaccacatttccctgtagagaatattagtgcagctcaaattacaatgtgcccccatgtgattgttgatgtgagacagcttgaacctgtgcttttgcccctccctgacataaggaacagattctttcattacaaccaggaagacaccccccggatgagacttgtggccatgttgtacacacctcttagagcaaactctggtgaggacgtgttcactgtgtcttgcagagtcttgacccgcccagcccctgattttgagttcacattcttagtgccaccaaccgtggaatcaaagactaagccttttacactccctattttaaccctaggggaactatccaattccagattccctgctccaatagacatgctgtacacagatcctaatgagacaattgtggtacaaccacaaaatggtagatgcaccctagatgggacactccaagggaccacccagctggtgcccacccaaatttgctcttttaggggcacgttgatcagccaaacgtcgaggtcagcagattcaacagactcagctccacgggtgaggaaccacccccttcacgttcagctgaagaacctcgacgggacaccatatgacccaacagatgaggtgccggcagttctgggtgccatagactttaaaggaactgtgtttggagtcgctagccagaggaacactacagggagctctgtaggggcgactcgtgcccatgaggtgcacatagacaccacaaaccctagatacaccccaaaacttggttctgtgttgatgcattctgagtctagtgattttgatgatggacaaccaacccgcttcacacccattggcatgggagcagatgattggcaccaatgggaattgcccgaatattcaggtcaccttactctcaacatgaacctagcccctgcagttgctcctgctttccccggtgagcgcatcctcttctttaggtcagtggttccatctgctggtggctacggatcaggccaaatagactgcctcatcccacaggagtgggttcagcacttctatcaggaggccgccccttcacaatctgcggtggctcttattagatatgttaaccctgacactgggagaaacatctttgaggcaaagctacacagagaagggttcattactgtggcaaattctggaaacaaccccatagttgtgcccccgaatggctattttaggtttgaggcctgggtcaatcaattctacacactcacccccatgggaactggacaggggcgcaggagagtccaataatggcaggagctttctttgcaggacttgcaggtgacgccataacgaatggtgtcgggtccctgatcaacgctggggccaatgcaatcaaccagaaggtggagtatgatttcaacaaacaactccaattggcatcttttaagcatgacaaggagatgctgcaatcacaagttctagccaccaaacaactccagcaggaaatgatgaacataaggcaaggggtcttgaccgctggcggcttttcccctactgatgccgcgaggggcgctgtaaacgcgccaatgacaaagatcctggattggaatggtacaagatattttgccccaaatagcatgaaaacaaccagttattcaggtcagttttccagtaatcctgtgcataggcaacccactttgtcccgtcctgattcccaaaaagtcaaaattaatagtgattctgctagtatatatagttctatgtctactgctccttcacaatcaacccattcaatgattctgacttcagggtctggatcgtccaggacaacctcctctcccacagtgacttccaccctatctaggaccagtgactgggtgagggggcaaaatgagaggcttagcccgttcatggatggtgctctccaaacaacttttgtcacaccaccatcgagcagagcttcatcaaatgggtcggtctcgaccgttcccaaagctgttttggactcctggactcctatgttcaatacccataggcagcctctcttcgctcacttgcgtaggcgaggggagtcacaaatttagtgaaaagattgatcaggttttcttcttccttctttctccttttctttctttt

SEQ ID NO: 434 - DNA, 1620 bp, Norovirus GII.17
atgaagatggcgtcgaatgacgccgctccatctaatgatggtgctgctggtctcgtaccagagggcaacaacgagacccttcccctagaaccagttgcgggcgcagctatagccgcacccgtcactggccaaaataatataattgacccctggattagaacaaattttgtgcaagcaccaaatggagagttcacagtgtcacccagaaactctcctggagaaattttattaaatttagagttgggccctgatttgaacccttatttggctcatttgtcaaggatgtacaatgggtatgctggtggagtggaagttcaggttctcctggcagggaacgcgttcactgccggaaagatcctcttcgccgccgtcccgccaaatttcccagtggaattcttaagcccggcccagatcacaatgctcccacatttaatagtagatgttaggactcttgaaccaattatgatcccactccctgatgttaggaatacattcttccattatagtaaccagcctaacagccgcatgagattagtggctatgctctataccccactcagatctaatggctcaggtgatgatgtctttactgtctcttgcagggttttgactaggcctactcctgattttgagttcacttatttagtgccaccttctgttgaatctaaaactaagcctttttccttacctattttaaccctttctgagctcacaaattcgaggtttccagtccccatcgattcgcttttcaccgcccagaataatgtgttgcaggtgcagtgtcaaaatggcaggtgtacacttgatggtgagttacaaggcacaacccagttgctcccaactggcatctgtgcattcagaggacgggtgacagcacaaattaaccaacgtgacaggtggcacatgcaactgcaaaacctcaatggtacaacatatgacccaactgatgatgtgccagccccgctgggtacacctgacttcaagggcgtcgtgtttgggatggtaagccaaagaaatgtgggtaatgatgcgcctggctcaaccagagcccaacaggcgtgggtttcaacctatagcccccaatttgtccccaaattaggttctgtcaatcttagaattagtgataatgatgatttccaattccagccgacaaaattcacaccagtgggcgtcaatgatgacgatgatggccacccgttcagacaatgggaactaccaaactattcaggggagcttaccttgaatatgaatcttgcccccccagttgctccaaattttcctggtgaacaattgttattcttcagatctttcgtgccatgctcaggaggttacaaccaaggtattatagattgtcttattccccaagaatggatccaacacttctatcaggaatcagcaccctcccagtcagacgtggccctaatcaggtatgtcaaccccgatacgggacgtacactgtttgaagcaaaattgcacagatctggttacattactgtggctcactctggagactatcctcttgttgttccggctaatggacactttagatttgattcttgggtaaatcagttttactcactcgccccaatgggaactgggaatgggcgaaggagggctcag